European Patent Application EP 4 653 447 A1, published November 26, 2025. Title: MODIFIED NUCLEOSIDE MONOMER AND DOUBLE-STRANDED RIBONUCLEIC ACID. Applicant: CSPC Zhongqi Pharmaceutical Technology (Shijiazhuang) Co., Ltd. Application CN. The sequence listing filed with the application follows.

SEQUENCE LISTING (77 sequences)

SEQ ID NO: 1 - RNA, 21 nt, synthetic construct
  source 1..21: mol_type = other RNA
aatgacttttattgagctctt

SEQ ID NO: 2 - RNA, 23 nt, synthetic construct
  source 1..23: mol_type = other RNA
  modified_base 6: mod_base = OTHER; note = M3C,2M4C,M4C,OR CP4C
aagagntcaataaaagtcattct

SEQ ID NO: 3 - RNA, 23 nt, synthetic construct
  source 1..23: mol_type = other RNA
  modified_base 8: mod_base = OTHER; note = M3C,2M4C,M4C,OR CP4C
aagagctnaataaaagtcattct

SEQ ID NO: 4 - RNA, 21 nt, synthetic construct
  source 1..21: mol_type = other RNA
ccacaacgcttttgggggtga

SEQ ID NO: 5 - RNA, 23 nt, synthetic construct
  source 1..23: mol_type = other RNA
  modified_base 6: mod_base = OTHER; note = M3C,2M4C,M4C,OR CP4C
tcaccnccaaaagcgttgtgggc

SEQ ID NO: 6 - RNA, 23 nt, synthetic construct
  source 1..23: mol_type = other RNA
  modified_base 7: mod_base = OTHER; note = M3C,2M4C,M4C,OR CP4C
tcacccncaaaagcgttgtgggc

SEQ ID NO: 7 - RNA, 23 nt, synthetic construct
  source 1..23: mol_type = other RNA
  modified_base 8: mod_base = OTHER; note = M3C,2M4C,M4C,OR CP4C
tcaccccnaaaagcgttgtgggc

SEQ ID NO: 8 - RNA, 21 nt, synthetic construct
  source 1..21: mol_type = other RNA
gagaattttggttgggcctag

SEQ ID NO: 9 - RNA, 23 nt, synthetic construct
  source 1..23: mol_type = other RNA
  modified_base 6: mod_base = OTHER; note = M3C,2M4C,M4C,OR CP4C
ctaggnccaaccaaaattctcca

SEQ ID NO: 10 - RNA, 23 nt, synthetic construct
  source 1..23: mol_type = other RNA
  modified_base 7: mod_base = OTHER; note = M3C,2M4C,M4C,OR CP4C
ctaggcncaaccaaaattctcca

SEQ ID NO: 11 - RNA, 23 nt, synthetic construct
  source 1..23: mol_type = other RNA
  modified_base 8: mod_base = OTHER; note = M3C,2M4C,M4C,OR CP4C
ctaggccnaaccaaaattctcca

SEQ ID NO: 12 - RNA, 21 nt, synthetic construct
  source 1..21: mol_type = other RNA
cccagtgtcaggtgggagtac

SEQ ID NO: 13 - RNA, 23 nt, synthetic construct
  source 1..23: mol_type = other RNA
  modified_base 6: mod_base = OTHER; note = M3C,2M4C,M4C,OR CP4C
gtactnccacctgacactgggat

SEQ ID NO: 14 - RNA, 23 nt, synthetic construct
  source 1..23: mol_type = other RNA
  modified_base 7: mod_base = OTHER; note = M3C,2M4C,M4C,OR CP4C
gtactcncacctgacactgggat

SEQ ID NO: 15 - RNA, 23 nt, synthetic construct
  source 1..23: mol_type = other RNA
  modified_base 8: mod_base = OTHER; note = M3C,2M4C,M4C,OR CP4C
gtactccnacctgacactgggat

SEQ ID NO: 16 - RNA, 21 nt, synthetic construct
  source 1..21: mol_type = other RNA
gtgattcaagtttatggatac

SEQ ID NO: 17 - RNA, 23 nt, synthetic construct
  source 1..23: mol_type = other RNA
  modified_base 6: mod_base = OTHER; note = M3C,2M4C,M4C,OR CP4C
gtatcnataaacttgaatcacaa

SEQ ID NO: 18 - RNA, 21 nt, synthetic construct
  source 1..21: mol_type = other RNA
tgtgtatttggaagttgtatc

SEQ ID NO: 19 - RNA, 23 nt, synthetic construct
  source 1..23: mol_type = other RNA
  modified_base 8: mod_base = OTHER; note = M3C,2M4C,M4C,OR CP4C
gatacaanttccaaatacacata

SEQ ID NO: 20 - RNA, 21 nt, synthetic construct
  source 1..21: mol_type = other RNA
gtgaagaaatgttgttacgat

SEQ ID NO: 21 - RNA, 23 nt, synthetic construct
  source 1..23: mol_type = other RNA
  modified_base 8: mod_base = OTHER; note = M3C,2M4C,M4C,OR CP4C
atcgtaanaacatttcttcacta

SEQ ID NO: 22 - RNA, 21 nt, synthetic construct
  source 1..21: mol_type = other RNA
aatgacttttattgagctctt

SEQ ID NO: 23 - RNA, 23 nt, synthetic construct
  source 1..23: mol_type = other RNA
  modified_base 6: mod_base = OTHER; note = M3C,2M4C,M4C,OR CP4C
aagagntcaataaaagtcattct

SEQ ID NO: 24 - RNA, 23 nt, synthetic construct
  source 1..23: mol_type = other RNA
  modified_base 8: mod_base = OTHER; note = M3C,2M4C,M4C,OR CP4C
aagagctnaataaaagtcattct

SEQ ID NO: 25 - RNA, 21 nt, synthetic construct
  source 1..21: mol_type = other RNA
ccacaacgcttttgggggtga

SEQ ID NO: 26 - RNA, 23 nt, synthetic construct
  source 1..23: mol_type = other RNA
  modified_base 6: mod_base = OTHER; note = M3C,2M4C,M4C,OR CP4C
tcaccnccaaaagcgttgtgggc

SEQ ID NO: 27 - RNA, 23 nt, synthetic construct
  source 1..23: mol_type = other RNA
  modified_base 7: mod_base = OTHER; note = M3C,2M4C,M4C,OR CP4C
tcacccncaaaagcgttgtgggc

SEQ ID NO: 28 - RNA, 23 nt, synthetic construct
  source 1..23: mol_type = other RNA
  modified_base 8: mod_base = OTHER; note = M3C,2M4C,M4C,OR CP4C
tcaccccnaaaagcgttgtgggc

SEQ ID NO: 29 - RNA, 21 nt, synthetic construct
  source 1..21: mol_type = other RNA
gagaattttggttgggcctag

SEQ ID NO: 30 - RNA, 23 nt, synthetic construct
  source 1..23: mol_type = other RNA
  modified_base 6: mod_base = OTHER; note = M3C,2M4C,M4C,OR CP4C
ctaggnccaaccaaaattctcca

SEQ ID NO: 31 - RNA, 23 nt, synthetic construct
  source 1..23: mol_type = other RNA
  modified_base 7: mod_base = OTHER; note = M3C,2M4C,M4C,OR CP4C
ctaggcncaaccaaaattctcca

SEQ ID NO: 32 - RNA, 23 nt, synthetic construct
  source 1..23: mol_type = other RNA
  modified_base 8: mod_base = OTHER; note = M3C,2M4C,M4C,OR CP4C
ctaggccnaaccaaaattctcca

SEQ ID NO: 33 - RNA, 21 nt, synthetic construct
  source 1..21: mol_type = other RNA
cccagtgtcaggtgggagtac

SEQ ID NO: 34 - RNA, 23 nt, synthetic construct
  source 1..23: mol_type = other RNA
  modified_base 6: mod_base = OTHER; note = M3C,2M4C,M4C,OR CP4C
gtactnccacctgacactgggat

SEQ ID NO: 35 - RNA, 23 nt, synthetic construct
  source 1..23: mol_type = other RNA
  modified_base 7: mod_base = OTHER; note = M3C,2M4C,M4C,OR CP4C
gtactcncacctgacactgggat

SEQ ID NO: 36 - RNA, 23 nt, synthetic construct
  source 1..23: mol_type = other RNA
  modified_base 8: mod_base = OTHER; note = M3C,2M4C,M4C,OR CP4C
gtactccnacctgacactgggat

SEQ ID NO: 37 - RNA, 21 nt, synthetic construct
  source 1..21: mol_type = other RNA
gtgattcaagtttatggatac

SEQ ID NO: 38 - RNA, 23 nt, synthetic construct
  source 1..23: mol_type = other RNA
  modified_base 6: mod_base = OTHER; note = M3C,2M4C,M4C,OR CP4C
gtatcnataaacttgaatcacaa

SEQ ID NO: 39 - RNA, 21 nt, synthetic construct
  source 1..21: mol_type = other RNA
tgtgtatttggaagttgtatc

SEQ ID NO: 40 - RNA, 23 nt, synthetic construct
  source 1..23: mol_type = other RNA
  modified_base 8: mod_base = OTHER; note = M3C,2M4C,M4C,OR CP4C
gatacaanttccaaatacacata

SEQ ID NO: 41 - RNA, 21 nt, synthetic construct
  source 1..21: mol_type = other RNA
gtgaagaaatgttgttacgat

SEQ ID NO: 42 - RNA, 23 nt, synthetic construct
  source 1..23: mol_type = other RNA
  modified_base 8: mod_base = OTHER; note = M3C,2M4C,M4C,OR CP4C
atcgtaanaacatttcttcacta

SEQ ID NO: 43 - RNA, 21 nt, synthetic construct
  source 1..21: mol_type = other RNA
ttctccgaacgtgtcacgttt

SEQ ID NO: 44 - RNA, 21 nt, synthetic construct
  source 1..21: mol_type = other RNA
acgtgacacgttcggagaatt

SEQ ID NO: 45 - RNA, 23 nt, synthetic construct
  source 1..23: mol_type = other RNA
aagagctcaataaaagtcattct

SEQ ID NO: 46 - RNA, 23 nt, synthetic construct
  source 1..23: mol_type = other RNA
  modified_base 6: mod_base = m3c
aagagntcaataaaagtcattct

SEQ ID NO: 47 - RNA, 23 nt, synthetic construct
  source 1..23: mol_type = other RNA
  modified_base 8: mod_base = m3c
aagagctnaataaaagtcattct

SEQ ID NO: 48 - RNA, 23 nt, synthetic construct
  source 1..23: mol_type = other RNA
  modified_base 6: mod_base = OTHER; note = 2M4C
aagagntcaataaaagtcattct

SEQ ID NO: 49 - RNA, 23 nt, synthetic construct
  source 1..23: mol_type = other RNA
  modified_base 6: mod_base = m4c
aagagntcaataaaagtcattct

SEQ ID NO: 50 - RNA, 23 nt, synthetic construct
  source 1..23: mol_type = other RNA
  modified_base 8: mod_base = m4c
aagagctnaataaaagtcattct

SEQ ID NO: 51 - RNA, 23 nt, synthetic construct
  source 1..23: mol_type = other RNA
  modified_base 6: mod_base = OTHER; note = CP4C
aagagntcaataaaagtcattct

SEQ ID NO: 52 - RNA, 23 nt, synthetic construct
  source 1..23: mol_type = other RNA
  modified_base 8: mod_base = OTHER; note = CP4C
aagagctnaataaaagtcattct

SEQ ID NO: 53 - RNA, 23 nt, synthetic construct
  source 1..23: mol_type = other RNA
tcacccccaaaagcgttgtgggc

SEQ ID NO: 54 - RNA, 23 nt, synthetic construct
  source 1..23: mol_type = other RNA
  modified_base 6: mod_base = OTHER; note = 2M4C
tcaccnccaaaagcgttgtgggc

SEQ ID NO: 55 - RNA, 23 nt, synthetic construct
  source 1..23: mol_type = other RNA
  modified_base 7: mod_base = OTHER; note = 2M4C
tcacccncaaaagcgttgtgggc

SEQ ID NO: 56 - RNA, 23 nt, synthetic construct
  source 1..23: mol_type = other RNA
  modified_base 6: mod_base = OTHER; note = CP4C
tcaccnccaaaagcgttgtgggc

SEQ ID NO: 57 - RNA, 23 nt, synthetic construct
  source 1..23: mol_type = other RNA
  modified_base 7: mod_base = OTHER; note = CP4C
tcacccncaaaagcgttgtgggc

SEQ ID NO: 58 - RNA, 23 nt, synthetic construct
  source 1..23: mol_type = other RNA
  modified_base 8: mod_base = OTHER; note = CP4C
tcaccccnaaaagcgttgtgggc

SEQ ID NO: 59 - RNA, 23 nt, synthetic construct
  source 1..23: mol_type = other RNA
  modified_base 6: mod_base = OTHER; note = 2M4C
tcaccnccaaaagcgttgtgggc

SEQ ID NO: 60 - RNA, 23 nt, synthetic construct
  source 1..23: mol_type = other RNA
  modified_base 7: mod_base = OTHER; note = 2M4C
tcacccncaaaagcgttgtgggc

SEQ ID NO: 61 - RNA, 23 nt, synthetic construct
  source 1..23: mol_type = other RNA
ctaggcccaaccaaaattctcca

SEQ ID NO: 62 - RNA, 23 nt, synthetic construct
  source 1..23: mol_type = other RNA
  modified_base 6: mod_base = OTHER; note = 2M4C
ctaggnccaaccaaaattctcca

SEQ ID NO: 63 - RNA, 23 nt, synthetic construct
  source 1..23: mol_type = other RNA
  modified_base 6: mod_base = OTHER; note = 2M4C
ctaggcncaaccaaaattctcca

SEQ ID NO: 64 - RNA, 23 nt, synthetic construct
  source 1..23: mol_type = other RNA
  modified_base 6: mod_base = OTHER; note = CP4C
ctaggnccaaccaaaattctcca

SEQ ID NO: 65 - RNA, 23 nt, synthetic construct
  source 1..23: mol_type = other RNA
  modified_base 7: mod_base = OTHER; note = CP4C
ctaggcncaaccaaaattctcca

SEQ ID NO: 66 - RNA, 23 nt, synthetic construct
  source 1..23: mol_type = other RNA
  modified_base 8: mod_base = OTHER; note = CP4C
ctaggccnaaccaaaattctcca

SEQ ID NO: 67 - RNA, 23 nt, synthetic construct
  source 1..23: mol_type = other RNA
gtactcccacctgacactgggat

SEQ ID NO: 68 - RNA, 23 nt, synthetic construct
  source 1..23: mol_type = other RNA
  modified_base 6: mod_base = OTHER; note = 2M4C
gtactnccacctgacactgggat

SEQ ID NO: 69 - RNA, 23 nt, synthetic construct
  source 1..23: mol_type = other RNA
  modified_base 6: mod_base = OTHER; note = CP4C
gtactnccacctgacactgggat

SEQ ID NO: 70 - RNA, 23 nt, synthetic construct
  source 1..23: mol_type = other RNA
  modified_base 7: mod_base = OTHER; note = CP4C
gtactcncacctgacactgggat

SEQ ID NO: 71 - RNA, 23 nt, synthetic construct
  source 1..23: mol_type = other RNA
  modified_base 8: mod_base = OTHER; note = CP4C
gtactccnacctgacactgggat

SEQ ID NO: 72 - RNA, 23 nt, synthetic construct
  source 1..23: mol_type = other RNA
gtatccataaacttgaatcacaa

SEQ ID NO: 73 - RNA, 23 nt, synthetic construct
  source 1..23: mol_type = other RNA
  modified_base 6: mod_base = OTHER; note = 2M4C
gtatcnataaacttgaatcacaa

SEQ ID NO: 74 - RNA, 23 nt, synthetic construct
  source 1..23: mol_type = other RNA
gatacaacttccaaatacacata

SEQ ID NO: 75 - RNA, 23 nt, synthetic construct
  source 1..23: mol_type = other RNA
  modified_base 8: mod_base = OTHER; note = CP4C
gatacaanttccaaatacacata

SEQ ID NO: 76 - RNA, 23 nt, synthetic construct
  source 1..23: mol_type = other RNA
atcgtaacaacatttcttcacta

SEQ ID NO: 77 - RNA, 23 nt, synthetic construct
  source 1..23: mol_type = other RNA
  modified_base 8: mod_base = OTHER; note = 2M4C
atcgtaanaacatttcttcacta